European Patent Application EP 4 338 745 A1, published March 20, 2024. Title: Allogeneic Human Macrophages for Cell Therapy. Applicant: Technische Universität Dresden. The sequence listing filed with the application follows.

SEQUENCE LISTING (20 sequences)

SEQ ID NO: 1 - DNA, 99 bp, Homo sapiens
  source 1..99: mol_type = other DNA
atctggcggagcggcggcgggttttagagctagaaatagcaagttaaaataaggctagtccgttatcaacttgaaaaagtggcaccgagtcggtgcttt

SEQ ID NO: 2 - DNA, 99 bp, Homo sapiens
  source 1..99: mol_type = other DNA
accctgataagtgctccgcggttttagagctagaaatagcaagttaaaataaggctagtccgttatcaacttgaaaaagtggcaccgagtcggtgcttt

SEQ ID NO: 3 - DNA, 99 bp, Homo sapiens
  source 1..99: mol_type = other DNA
cggccgcaaagtttcccggggttttagagctagaaatagcaagttaaaataaggctagtccgttatcaacttgaaaaagtggcaccgagtcggtgcttt

SEQ ID NO: 4 - DNA, 99 bp, Homo sapiens
  source 1..99: mol_type = other DNA
tgacctgtttgacttgagcggttttagagctagaaatagcaagttaaaataaggctagtccgttatcaacttgaaaaagtggcaccgagtcggtgcttt

SEQ ID NO: 5 - DNA, 99 bp, synthetic construct
  source 1..99: mol_type = other DNA
  misc_feature 1..20: note = n can be a, g, c or t
nnnnnnnnnnnnnnnnnnnngttttagagctagaaatagcaagttaaaataaggctagtccgttatcaacttgaaaaagtggcaccgagtcggtgcttt

SEQ ID NO: 6 - DNA, 20 bp, Homo sapiens
  source 1..20: mol_type = other DNA
atctggcggagcggcggcgg

SEQ ID NO: 7 - DNA, 20 bp, Homo sapiens
  source 1..20: mol_type = other DNA
accctgataagtgctccgcg

SEQ ID NO: 8 - DNA, 20 bp, Homo sapiens
  source 1..20: mol_type = other DNA
cggccgcaaagtttcccggg

SEQ ID NO: 9 - DNA, 20 bp, Homo sapiens
  source 1..20: mol_type = other DNA
tgacctgtttgacttgagcg

SEQ ID NO: 10 - DNA, 45 bp, Homo sapiens
  source 1..45: mol_type = other DNA
atctggcggagcggcggcggcggcggcggcggcggcaggagaatg

SEQ ID NO: 11 - DNA, 48 bp, Homo sapiens
  source 1..48: mol_type = other DNA
tgagtctgacacgcgattccagctagccaccctgataagtgctccgcg

SEQ ID NO: 12 - DNA, 53 bp, Homo sapiens
  source 1..53: mol_type = other DNA
cggccgcaaagtttcccgggcggcagcggcggctgcgcctcgcttcagcgatg

SEQ ID NO: 13 - DNA, 17 bp, synthetic construct
  source 1..17: mol_type = other DNA
cggccgcaaagtttccc

SEQ ID NO: 14 - DNA, 10 bp, synthetic construct
  source 1..10: mol_type = other DNA
cggccgcaaa

SEQ ID NO: 15 - DNA, 15 bp, synthetic construct
  source 1..15: mol_type = other DNA
cggccgcaaagtttc

SEQ ID NO: 16 - DNA, 14 bp, synthetic construct
  source 1..14: mol_type = other DNA
cggccgcaaagttt

SEQ ID NO: 17 - DNA, 23 bp, synthetic construct
  source 1..23: mol_type = other DNA
ccttgacctgtttgacttgagcg

SEQ ID NO: 18 - DNA, 17 bp, synthetic construct
  source 1..17: mol_type = other DNA
cctgtttgacttgagcg

SEQ ID NO: 19 - DNA, 14 bp, synthetic construct
  source 1..14: mol_type = other DNA
ctttgacttgagcg

SEQ ID NO: 20 - DNA, 18 bp, synthetic construct
  source 1..18: mol_type = other DNA
tcctgtttgacttgagcg